European Patent Specification EP 3 622 082 B1, published March 29, 2023. Title: Method for detecting C. perfringens induced diseases in animals. Applicant: Evonik Degussa GmbH. The sequence listing filed with the application follows.

SEQUENCE LISTING (16 sequences)

SEQ ID NO: 1 - DNA, 969 bp, Clostridium perfringens
  misc_feature (10)..(10): n is a, c, g, or t
  misc_feature (391)..(396): n is a, c, g, or t
  misc_feature (418)..(420): n is a, c, g, or t
  misc_feature (443)..(443): n is a, c, g, or t
  misc_feature (497)..(497): n is a, c, g, or t
  misc_feature (502)..(502): n is a, c, g, or t
ttgaaaagantaaaaattatttcaattacactagttcttacaagtgtaattagtacaagccttttttcaactcaaactcaagtttttgcaagtgaattaaatgacataaacaaaattgagttgaaaaatctaagtggagaaataataaaagaaaatggaaaggaagctattaaatatacttctagtgataccgcttcacataaaggttggaaggcaactttaagtggaacatttattgaagatcctcattctgataagaaaactgctttattaaatttagaaggatttataccttctgataaacagatttttggttctaaatattacggaaaaatgaaatggcctgaaacttatagaattaatgtaaaaagtgctgatgtaaataataatnnnnnnatagcaaattctattcctaaannnactatagataaaaaagatgtatntaattcaattggttattctataggcggtaatatatctgttgaaggaaaaactgntggtnctggaataaatgcttcatataatgtccaaaatactataagctatgaacaacctgattttagaacaattcaaagaaaagatgatgcaaatttagcatcatgggatataaaatttgttgagactaaggacggttataatatagattcttatcatgctatttatggaaatcaattattcatgaaatcaagattgtataataatggtgataaaaatttcacagatgatagagatttatcaacattaatttctggtggattttcacccaatatggctttagcattaacagcacctaaaaatgctaaagaatctgtaataatagttgaatatcaaagatttgataatgactatattttaaattgggaaactactcaatggcgaggaacaaacaaactttcgtcaacaagtgaatataacgaatttatgtttaaaataaattggcaagatcataaaatagaatattatctgtaa

SEQ ID NO: 2 - DNA, 1197 bp, Clostridium perfringens
  misc_feature (21)..(21): n is a, c, g, or t
  misc_feature (23)..(24): n is a, c, g, or t
  misc_feature (28)..(28): n is a, c, g, or t
  misc_feature (36)..(37): n is a, c, g, or t
  misc_feature (40)..(40): n is a, c, g, or t
  misc_feature (44)..(44): n is a, c, g, or t
  misc_feature (64)..(65): n is a, c, g, or t
  misc_feature (78)..(78): n is a, c, g, or t
  misc_feature (81)..(81): n is a, c, g, or t
  misc_feature (96)..(96): n is a, c, g, or t
  misc_feature (102)..(102): n is a, c, g, or t
  misc_feature (128)..(128): n is a, c, g, or t
  misc_feature (138)..(139): n is a, c, g, or t
  misc_feature (147)..(147): n is a, c, g, or t
  misc_feature (160)..(160): n is a, c, g, or t
  misc_feature (165)..(165): n is a, c, g, or t
  misc_feature (167)..(167): n is a, c, g, or t
  misc_feature (170)..(170): n is a, c, g, or t
  misc_feature (213)..(213): n is a, c, g, or t
  misc_feature (225)..(225): n is a, c, g, or t
  misc_feature (264)..(264): n is a, c, g, or t
  misc_feature (267)..(267): n is a, c, g, or t
  misc_feature (274)..(274): n is a, c, g, or t
  misc_feature (288)..(288): n is a, c, g, or t
  misc_feature (307)..(307): n is a, c, g, or t
  misc_feature (318)..(318): n is a, c, g, or t
  misc_feature (360)..(360): n is a, c, g, or t
  misc_feature (393)..(393): n is a, c, g, or t
  misc_feature (420)..(420): n is a, c, g, or t
  misc_feature (423)..(423): n is a, c, g, or t
  misc_feature (429)..(429): n is a, c, g, or t
  misc_feature (453)..(453): n is a, c, g, or t
  misc_feature (510)..(510): n is a, c, g, or t
  misc_feature (540)..(540): n is a, c, g, or t
  misc_feature (552)..(552): n is a, c, g, or t
  misc_feature (558)..(558): n is a, c, g, or t
  misc_feature (567)..(567): n is a, c, g, or t
  misc_feature (584)..(584): n is a, c, g, or t
  misc_feature (600)..(600): n is a, c, g, or t
  misc_feature (604)..(605): n is a, c, g, or t
  misc_feature (613)..(613): n is a, c, g, or t
  misc_feature (621)..(621): n is a, c, g, or t
  misc_feature (633)..(633): n is a, c, g, or t
  misc_feature (680)..(680): n is a, c, g, or t
  misc_feature (684)..(684): n is a, c, g, or t
  misc_feature (738)..(738): n is a, c, g, or t
  misc_feature (741)..(742): n is a, c, g, or t
  misc_feature (757)..(757): n is a, c, g, or t
  misc_feature (759)..(759): n is a, c, g, or t
  misc_feature (783)..(783): n is a, c, g, or t
  misc_feature (807)..(807): n is a, c, g, or t
  misc_feature (825)..(826): n is a, c, g, or t
  misc_feature (840)..(840): n is a, c, g, or t
  misc_feature (843)..(843): n is a, c, g, or t
  misc_feature (885)..(885): n is a, c, g, or t
  misc_feature (963)..(963): n is a, c, g, or t
  misc_feature (978)..(978): n is a, c, g, or t
  misc_feature (985)..(985): n is a, c, g, or t
  misc_feature (993)..(993): n is a, c, g, or t
  misc_feature (999)..(999): n is a, c, g, or t
  misc_feature (1014)..(1014): n is a, c, g, or t
  misc_feature (1020)..(1020): n is a, c, g, or t
  misc_feature (1087)..(1087): n is a, c, g, or t
  misc_feature (1094)..(1094): n is a, c, g, or t
  misc_feature (1117)..(1117): n is a, c, g, or t
  misc_feature (1124)..(1124): n is a, c, g, or t
  misc_feature (1143)..(1143): n is a, c, g, or t
  misc_feature (1149)..(1149): n is a, c, g, or t
  misc_feature (1158)..(1158): n is a, c, g, or t
atgaaaagaaagatttgtaangnncttntttgtgcnncgntagnaactagcctatgggctgggnnatcaactaaagtntangcttgggatggaaanattganggaacaggaactcatgctatgattgnaactcaaggnntttcaatnttagaaaatgatntgtcnanaantgaaccagaaagtgtaagaaaaaacttagagattttaaaaganaacatgcatgancttcaattaggttctacttatccagattatgataagaangcntatgatntatatcaagatcanttctgggatcctgatacanataataatttntcaaaggataatagttggtatttagcttattctatacctganacaggggaatcacaaataagaaaattttcagcnttagctagatatgaatggcaaagaggnaantataancaagctacattctatcttggagangctatgcactattttggagatatagatactccatatcatcctgctaatgttactgcngttgatagcgcaggacatgttaagtttganacttttgcagangaaagnaaagaacantataaaataaacacagnaggttgcaaaactaangagnntttttatnctgatatnttaaaaaacaangattttaatgcatggtcaaaagaatatgcaagaggttttgctaaaanaggnaaatcaatatactatagtcatgctagcatgagtcatagttgggatgattgggantanncagcaaaggtaactntngctaactctcaaaaaggaacagcnggatatatttatagattcttacangatgtatcagagggtaannatccatcagttggnaanaatgtaaaagaactagtagcttacatatcaactagtggtganaaagatgctggaacagatgactacatgtattttggaatcaaaacaaaggatggaaaaactcaagaatgggaaatgganaacccaggaaatgantttatgnctggaagnaaaganacttatactttcaanttaaangatgaaaatctaaaaattgatgatatacaaaatatgtggattagaaaaagaaaatatacagcattcncagatgnttataagccagaaaacataaagntaatagnaaatggaaaagttgtagtngacaangatataaangagtggatttcaggaaattcaacttataatataaaataa

SEQ ID NO: 3 - DNA, 20 bp, Artificial Sequence
  Primer
tatacttctagtgataccgc

SEQ ID NO: 4 - DNA, 20 bp, Artificial Sequence
  Primer
atcagaatgaggatcttcaa

SEQ ID NO: 5 - DNA, 23 bp, Artificial Sequence
  Probe
tcacataaaggttggaaggcaac

SEQ ID NO: 6 - DNA, 20 bp, Artificial Sequence
  Primer
tacatatcaactagtggtga

SEQ ID NO: 7 - DNA, 20 bp, Artificial Sequence
  Primer
attcttgagtttttccatcc

SEQ ID NO: 8 - DNA, 27 bp, Artificial Sequence
  Probe
tggaacagatgactacatgtattttgg

SEQ ID NO: 9 - DNA, 20 bp, Artificial Sequence
  Primer
agtctacgcttgggatggaa

SEQ ID NO: 10 - DNA, 20 bp, Artificial Sequence
  Primer
tttcctgggttgttcatttc

SEQ ID NO: 11 - DNA, 22 bp, Artificial Sequence
  Primer
tgataccgcttcacataaaggt

SEQ ID NO: 12 - DNA, 22 bp, Artificial Sequence
  Primer
accgtccttagtctcaacaaat

SEQ ID NO: 13 - DNA, 24 bp, Artificial Sequence
  Primer
gttgatagcgcaggacatgttaag

SEQ ID NO: 14 - DNA, 24 bp, Artificial Sequence
  Primer
catgtagtcatctgttccagcatc

SEQ ID NO: 15 - DNA, 25 bp, Artificial Sequence
  Primer
tcaattggttattctataggcggta

SEQ ID NO: 16 - DNA, 25 bp, Artificial Sequence
  Primer
atatgaagcatttattccagcacca